European Patent Application EP 4 582 540 A1, published July 9, 2025. Title: 核酸分子の製造方法. Applicant: 株式会社ジーンデザイン. Application JP. The sequence listing filed with the application follows.

SEQUENCE LISTING (243 sequences)

SEQ ID NO: 1 - RNA, 20 nt, synthetic construct
  source 1..20: mol_type = other RNA
ggaaattaggtgcgcttggc

SEQ ID NO: 2 - RNA, 15 nt, synthetic construct
  source 1..15: mol_type = other RNA
gttttagagctagaa

SEQ ID NO: 3 - RNA, 19 nt, synthetic construct
  source 1..19: mol_type = other RNA
atagcaagttaaaataagg

SEQ ID NO: 4 - RNA, 18 nt, synthetic construct
  source 1..18: mol_type = other RNA
ctagtccgttatcaactt

SEQ ID NO: 5 - RNA, 14 nt, synthetic construct
  source 1..14: mol_type = other RNA
gaaaaagtggcacc

SEQ ID NO: 6 - RNA, 14 nt, synthetic construct
  source 1..14: mol_type = other RNA
gagtcggtgctttt

SEQ ID NO: 7 - DNA, 27 bp, synthetic construct
  source 1..27: mol_type = other DNA
ctaaaacgccaagcgcacctaatttcc

SEQ ID NO: 8 - DNA, 22 bp, synthetic construct
  source 1..22: mol_type = other DNA
ttttaacttgctatttctagct

SEQ ID NO: 9 - DNA, 30 bp, synthetic construct
  source 1..30: mol_type = other DNA
ctttttcaagttgataacggactagcctta

SEQ ID NO: 10 - DNA, 21 bp, synthetic construct
  source 1..21: mol_type = other DNA
aaaagcaccgactcggtgcca

SEQ ID NO: 11 - DNA, 16 bp, synthetic construct
  source 1..16: mol_type = other DNA
tctaaaacgccaagcg

SEQ ID NO: 12 - DNA, 14 bp, synthetic construct
  source 1..14: mol_type = other DNA
ttgctatttctagc

SEQ ID NO: 13 - DNA, 18 bp, synthetic construct
  source 1..18: mol_type = other DNA
acggactagccttatttt

SEQ ID NO: 14 - DNA, 14 bp, synthetic construct
  source 1..14: mol_type = other DNA
ctttttcaagttga

SEQ ID NO: 15 - DNA, 14 bp, synthetic construct
  source 1..14: mol_type = other DNA
ccgactcggtgcca

SEQ ID NO: 16 - DNA, 100 bp, synthetic construct
  source 1..100: mol_type = other DNA
aaaagcaccgactcggtgccactttttcaagttgataacggactagccttattttaacttgctatttctagctctaaaacgccaagcgcacctaatttcc

SEQ ID NO: 17 - RNA, 20 nt, synthetic construct
  source 1..20: mol_type = other RNA
ggaaattaggtgcgcttggc

SEQ ID NO: 18 - RNA, 15 nt, synthetic construct
  source 1..15: mol_type = other RNA
gttttagagctagaa

SEQ ID NO: 19 - RNA, 19 nt, synthetic construct
  source 1..19: mol_type = other RNA
atagcaagttaaaataagg

SEQ ID NO: 20 - RNA, 18 nt, synthetic construct
  source 1..18: mol_type = other RNA
ctagtccgttatcaactt

SEQ ID NO: 21 - RNA, 14 nt, synthetic construct
  source 1..14: mol_type = other RNA
gaaaaagtggcacc

SEQ ID NO: 22 - RNA, 14 nt, synthetic construct
  source 1..14: mol_type = other RNA
gagtcggtgctttt

SEQ ID NO: 23 - RNA, 20 nt, synthetic construct
  source 1..20: mol_type = other RNA
  modified_base 1: mod_base = OTHER; note = 3-Phosphorothioated 2-OMe-G
  modified_base 2: mod_base = OTHER; note = 3-Phosphorothioated 2-OMe-G
  modified_base 3: mod_base = OTHER; note = 3-Phosphorothioated 2-OMe-A
nnnaattaggtgcgcttggc

SEQ ID NO: 24 - RNA, 14 nt, synthetic construct
  source 1..14: mol_type = other RNA
  modified_base 11: mod_base = OTHER; note = 3-Phosphorothioated U
  modified_base 12: mod_base = um
  modified_base 13: mod_base = OTHER; note = 3-Phosphorothioated 2-OMe- U
  modified_base 14: mod_base = um
gagtcggtgcnnnn

SEQ ID NO: 25 - RNA, 20 nt, synthetic construct
  source 1..20: mol_type = other RNA
  misc_feature 1..3: note = 3-Phosphorothioated
  misc_feature 15..16: note = 3-Phosphorothioated
  misc_feature 19: note = 3-Phosphorothioated
  modified_base 3..5: mod_base = OTHER; note = 2'-OMe
  modified_base 8: mod_base = OTHER; note = 2'-OMe
  modified_base 1..2: mod_base = gm
  modified_base 9..10: mod_base = gm
  modified_base 20: mod_base = cm
  modified_base 6..7: mod_base = um
  modified_base 11..14: mod_base = OTHER; note = 2'-F
  modified_base 17..18: mod_base = OTHER; note = 2'-F
ggaaattaggtgcgcttggc

SEQ ID NO: 26 - RNA, 15 nt, synthetic construct
  source 1..15: mol_type = other RNA
  misc_feature 2..4: note = 3-Phosphorothioated
  modified_base 8: mod_base = OTHER; note = 2'-OMe
  modified_base 12: mod_base = OTHER; note = 2'-OMe
  modified_base 14..15: mod_base = OTHER; note = 2'-OMe
  modified_base 1: mod_base = gm
  modified_base 7: mod_base = gm
  modified_base 9: mod_base = gm
  modified_base 13: mod_base = gm
  modified_base 10: mod_base = cm
  modified_base 11: mod_base = um
  modified_base 5..6: mod_base = OTHER; note = 2'-F
gttttagagctagaa

SEQ ID NO: 27 - RNA, 19 nt, synthetic construct
  source 1..19: mol_type = other RNA
  modified_base 1: mod_base = OTHER; note = 2'-OMe
  modified_base 3: mod_base = OTHER; note = 2'-OMe
  modified_base 6..7: mod_base = OTHER; note = 2'-OMe
  modified_base 11: mod_base = OTHER; note = 2'-OMe
  modified_base 13..14: mod_base = OTHER; note = 2'-OMe
  modified_base 16..17: mod_base = OTHER; note = 2'-OMe
  modified_base 4: mod_base = gm
  modified_base 8: mod_base = gm
  modified_base 18..19: mod_base = gm
  modified_base 5: mod_base = cm
  modified_base 2: mod_base = um
atagcaagttaaaataagg

SEQ ID NO: 28 - RNA, 18 nt, synthetic construct
  source 1..18: mol_type = other RNA
  modified_base 3: mod_base = OTHER; note = 2'-OMe
  modified_base 11: mod_base = OTHER; note = 2'-OMe
  modified_base 14..15: mod_base = OTHER; note = 2'-OMe
  modified_base 7: mod_base = cm
  modified_base 13: mod_base = cm
  modified_base 16: mod_base = cm
  modified_base 12: mod_base = um
  modified_base 17..18: mod_base = um
ctagtccgttatcaactt

SEQ ID NO: 29 - RNA, 14 nt, synthetic construct
  source 1..14: mol_type = other RNA
  modified_base 2..6: mod_base = OTHER; note = 2'-OMe
  modified_base 12: mod_base = OTHER; note = 2'-OMe
  modified_base 1: mod_base = gm
  modified_base 7: mod_base = gm
  modified_base 9..10: mod_base = gm
  modified_base 11: mod_base = cm
  modified_base 13..14: mod_base = cm
  modified_base 8: mod_base = um
gaaaaagtggcacc

SEQ ID NO: 30 - RNA, 14 nt, synthetic construct
  source 1..14: mol_type = other RNA
  misc_feature 10..13: note = 3-Phosphorothioated
  modified_base 2: mod_base = OTHER; note = 2'-OMe
  modified_base 1: mod_base = gm
  modified_base 3: mod_base = gm
  modified_base 6..7: mod_base = gm
  modified_base 9: mod_base = gm
  modified_base 5: mod_base = cm
  modified_base 10: mod_base = cm
  modified_base 4: mod_base = um
  modified_base 8: mod_base = um
  modified_base 11..14: mod_base = um
gagtcggtgctttt

SEQ ID NO: 31 - RNA, 19 nt, synthetic construct
  source 1..19: mol_type = other RNA
  modified_base 1: mod_base = OTHER; note = 2'-OMe
  modified_base 3: mod_base = OTHER; note = 2'-OMe
  modified_base 6..7: mod_base = OTHER; note = 2'-OMe
  modified_base 11: mod_base = OTHER; note = 2'-OMe
  modified_base 13..14: mod_base = OTHER; note = 2'-OMe
  modified_base 16..17: mod_base = OTHER; note = 2'-OMe
  modified_base 4: mod_base = gm
  modified_base 8: mod_base = gm
  modified_base 18..19: mod_base = gm
  modified_base 5: mod_base = cm
  modified_base 2: mod_base = um
  modified_base 9..10: mod_base = OTHER; note = 2'-F
  modified_base 12: mod_base = OTHER; note = 2'-F
  modified_base 15: mod_base = OTHER; note = 2'-F
atagcaagttaaaataagg

SEQ ID NO: 32 - RNA, 18 nt, synthetic construct
  source 1..18: mol_type = other RNA
  modified_base 3: mod_base = OTHER; note = 2'-OMe
  modified_base 11: mod_base = OTHER; note = 2'-OMe
  modified_base 14..15: mod_base = OTHER; note = 2'-OMe
  modified_base 7: mod_base = cm
  modified_base 13: mod_base = cm
  modified_base 16: mod_base = cm
  modified_base 12: mod_base = um
  modified_base 17..18: mod_base = um
  modified_base 1..2: mod_base = OTHER; note = 2'-F
  modified_base 4..6: mod_base = OTHER; note = 2'-F
  modified_base 8..10: mod_base = OTHER; note = 2'-F
ctagtccgttatcaactt

SEQ ID NO: 33 - RNA, 15 nt, synthetic construct
  source 1..15: mol_type = other RNA
  misc_feature 2..4: note = 3-Phosphorothioated
  modified_base 8: mod_base = OTHER; note = 2'-OMe
  modified_base 12: mod_base = OTHER; note = 2'-OMe
  modified_base 14..15: mod_base = OTHER; note = 2'-OMe
  modified_base 7: mod_base = gm
  modified_base 9: mod_base = gm
  modified_base 13: mod_base = gm
  modified_base 10: mod_base = cm
  modified_base 11: mod_base = um
  modified_base 5..6: mod_base = OTHER; note = 2'-F
  modified_base 1: mod_base = OTHER; note = LNA
gttttagagctagaa

SEQ ID NO: 34 - RNA, 15 nt, synthetic construct
  source 1..15: mol_type = other RNA
  misc_feature 2..4: note = 3-Phosphorothioated
  modified_base 8: mod_base = OTHER; note = 2'-OMe
  modified_base 12: mod_base = OTHER; note = 2'-OMe
  modified_base 14..15: mod_base = OTHER; note = 2'-OMe
  modified_base 7: mod_base = gm
  modified_base 9: mod_base = gm
  modified_base 13: mod_base = gm
  modified_base 10: mod_base = cm
  modified_base 11: mod_base = um
  modified_base 5..6: mod_base = OTHER; note = 2'-F
  modified_base 1: mod_base = OTHER; note = BNANC-Nme
gttttagagctagaa

SEQ ID NO: 35 - RNA, 15 nt, synthetic construct
  source 1..15: mol_type = other RNA
  misc_feature 2..4: note = 3-Phosphorothioated
  modified_base 8: mod_base = OTHER; note = 2'-OMe
  modified_base 12: mod_base = OTHER; note = 2'-OMe
  modified_base 14..15: mod_base = OTHER; note = 2'-OMe
  modified_base 7: mod_base = gm
  modified_base 9: mod_base = gm
  modified_base 13: mod_base = gm
  modified_base 10: mod_base = cm
  modified_base 11: mod_base = um
  modified_base 5..6: mod_base = OTHER; note = 2'-F
  modified_base 1: mod_base = OTHER; note = 2'-MOE
gttttagagctagaa

SEQ ID NO: 36 - DNA, 27 bp, synthetic construct
  source 1..27: mol_type = other DNA
ctaaaacgccaagcgcacctaatttcc

SEQ ID NO: 37 - DNA, 22 bp, synthetic construct
  source 1..22: mol_type = other DNA
ttttaacttgctatttctagct

SEQ ID NO: 38 - DNA, 30 bp, synthetic construct; identical to SEQ ID NO: 9
  source 1..30: mol_type = other DNA

SEQ ID NO: 39 - DNA, 21 bp, synthetic construct
  source 1..21: mol_type = other DNA
aaaagcaccgactcggtgcca

SEQ ID NO: 40 - RNA, 100 nt, synthetic construct
  source 1..100: mol_type = other RNA
ggaaattaggtgcgcttggcgttttagagctagaaatagcaagttaaaataaggctagtccgttatcaacttgaaaaagtggcaccgagtcggtgctttt

SEQ ID NO: 41 - RNA, 100 nt, synthetic construct
  source 1..100: mol_type = other RNA
  modified_base join(1,2): mod_base = OTHER; note = 3-Phosphorothioated 2-OMe-G
  modified_base 3: mod_base = OTHER; note = 3-Phosphorothioated 2-OMe-A
  modified_base 97: mod_base = OTHER; note = 3-Phosphorothioated U
  modified_base join(98,99): mod_base = OTHER; note = 3-Phosphorothioated 2-OMe-U
  modified_base 100: mod_base = um
nnnaattaggtgcgcttggcgttttagagctagaaatagcaagttaaaataaggctagtccgttatcaacttgaaaaagtggcaccgagtcggtgcnnnn

SEQ ID NO: 42 - RNA, 100 nt, synthetic construct
  source 1..100: mol_type = other RNA
  modified_base join(1,2): mod_base = OTHER; note = 3-Phosphorothioated 2-OMe-G
  modified_base 3: mod_base = OTHER; note = 3-Phosphorothioated 2-OMe-A
  modified_base join(4,5,8,28,32,34,35,36,38,41,42,46,48,49,51,52,57,65,68,69,74,75,76,77,78,84,88): mod_base = OTHER; note = 2-OMe-A
  modified_base join(6,7,31,37,66,71,72,80,90,94,100): mod_base = um
  modified_base join(9,10,21,27,29,33,39,43,53,54,73,79,81,82,87,89,92,93,95): mod_base = gm
  modified_base join(11,17,25): mod_base = OTHER; note = 2-Fluoro-U
  modified_base join(12,14,18): mod_base = OTHER; note = 2-Fluoro-G
  modified_base 13: mod_base = OTHER; note = 2-Fluoro-C
  modified_base 15: mod_base = OTHER; note = 3-Phosphorothioated C
  modified_base join(16,22,23,24): mod_base = OTHER; note = 3-Phosphorothioated U
  modified_base 19: mod_base = OTHER; note = 3-Phosphorothioated G
  modified_base join(20,30,40,61,67,70,83,85,86,91): mod_base = cm
  modified_base 96: mod_base = OTHER; note = 3-Phosphorothioated 2-OMe-C
  modified_base join(97,98,99): mod_base = OTHER; note = 3-Phosphorothioated 2-OMe-U
nnnnnnnnnnnnnnnnnnnnnnnnnnnnnnnnnnnnnnnnnnnttnanntnnnnctngtcngttnnnnnnnnnnnnnnnnnnnnnnnnnnnnnnnnnnnn

SEQ ID NO: 43 - RNA, 100 nt, synthetic construct; identical to SEQ ID NO: 40
  source 1..100: mol_type = other RNA
  misc_feature 1..3: note = 3-Phosphorothioated
  misc_feature 15..16: note = 3-Phosphorothioated
  misc_feature 19: note = 3-Phosphorothioated
  misc_feature 22..24: note = 3-Phosphorothioated
  misc_feature 96..99: note = 3-Phosphorothioated
  modified_base 3..5: mod_base = OTHER; note = 2'-OMe
  modified_base 8: mod_base = OTHER; note = 2'-OMe
  modified_base 28: mod_base = OTHER; note = 2'-OMe
  modified_base 32: mod_base = OTHER; note = 2'-OMe
  modified_base 34..36: mod_base = OTHER; note = 2'-OMe
  modified_base 38: mod_base = OTHER; note = 2'-OMe
  modified_base 41..42: mod_base = OTHER; note = 2'-OMe
  modified_base 46: mod_base = OTHER; note = 2'-OMe
  modified_base 48..49: mod_base = OTHER; note = 2'-OMe
  modified_base 51..52: mod_base = OTHER; note = 2'-OMe
  modified_base 57: mod_base = OTHER; note = 2'-OMe
  modified_base 65: mod_base = OTHER; note = 2'-OMe
  modified_base 68..69: mod_base = OTHER; note = 2'-OMe
  modified_base 74..78: mod_base = OTHER; note = 2'-OMe
  modified_base 84: mod_base = OTHER; note = 2'-OMe
  modified_base 88: mod_base = OTHER; note = 2'-OMe
  modified_base 1..2: mod_base = gm
  modified_base 9..10: mod_base = gm
  modified_base 21: mod_base = gm
  modified_base 27: mod_base = gm
  modified_base 29: mod_base = gm
  modified_base 33: mod_base = gm
  modified_base 39: mod_base = gm
  modified_base 43: mod_base = gm
  modified_base 53..54: mod_base = gm
  modified_base 73: mod_base = gm
  modified_base 79: mod_base = gm
  modified_base 81..82: mod_base = gm
  modified_base 87: mod_base = gm
  modified_base 89: mod_base = gm
  modified_base 92..93: mod_base = gm
  modified_base 95: mod_base = gm
  modified_base 20: mod_base = cm
  modified_base 30: mod_base = cm
  modified_base 40: mod_base = cm
  modified_base 61: mod_base = cm
  modified_base 67: mod_base = cm
  modified_base 70: mod_base = cm
  modified_base 83: mod_base = cm
  modified_base 85..86: mod_base = cm
  modified_base 91: mod_base = cm
  modified_base 96: mod_base = cm
  modified_base 6..7: mod_base = um
  modified_base 31: mod_base = um
  modified_base 37: mod_base = um
  modified_base 66: mod_base = um
  modified_base 71..72: mod_base = um
  modified_base 80: mod_base = um
  modified_base 90: mod_base = um
  modified_base 94: mod_base = um
  modified_base 97..100: mod_base = um
  modified_base 11..14: mod_base = OTHER; note = 2'-F
  modified_base 17..18: mod_base = OTHER; note = 2'-F
  modified_base 25..26: mod_base = OTHER; note = 2'-F
  modified_base 44..45: mod_base = OTHER; note = 2'-F
  modified_base 47: mod_base = OTHER; note = 2'-F
  modified_base 50: mod_base = OTHER; note = 2'-F
  modified_base 55..56: mod_base = OTHER; note = 2'-F
  modified_base 58..60: mod_base = OTHER; note = 2'-F
  modified_base 62..64: mod_base = OTHER; note = 2'-F

SEQ ID NO: 44 - RNA, 100 nt, synthetic construct
  source 1..100: mol_type = other RNA
  modified_base join(1,2): mod_base = OTHER; note = 3-Phosphorothioated 2-OMe-G
  modified_base 3: mod_base = OTHER; note = 3-Phosphorothioated 2-OMe-A
  modified_base join(4,5,8,28,32,34,35,38,46,49,50,55,56,57,58,59,65,69,82,84,87,88,92,94,95,97,98): mod_base = OTHER; note = 2-OMe-A
  modified_base join(6,7,31,47,52,53,61,71,75,81,83): mod_base = um
  modified_base join(9,10,27,29,33,54,60,62,63,68,70,73,74,76,85,89,99,100): mod_base = gm
  modified_base join(11,17,25,90,91,96): mod_base = OTHER; note = 2-Fluoro-U
  modified_base join(12,14,18): mod_base = OTHER; note = 2-Fluoro-G
  modified_base 13: mod_base = OTHER; note = 2-Fluoro-C
  modified_base 15: mod_base = OTHER; note = 3-Phosphorothioated C
  modified_base join(16,22,23,24): mod_base = OTHER; note = 3-Phosphorothioated U
  modified_base 19: mod_base = OTHER; note = 3-Phosphorothioated G
  modified_base join(20,30,42,48,51,64,66,67,72,86): mod_base = cm
  modified_base 77: mod_base = OTHER; note = 3-Phosphorothioated 2-OMe-C
  modified_base join(78,79,80): mod_base = OTHER; note = 3-Phosphorothioated 2-OMe-U
  modified_base join(26,93): mod_base = OTHER; note = 2-Fluoro-A
  modified_base 21: mod_base = OTHER; note = LNA-G
nnnnnnnnnnnnnnnnnnnnnnnnnnnnnnnnnnnctngtcngttnnnnnnnnnnnnnnnnnnnnnnnnnnnnnnnnnnnnnnnnnnnnttnanntnnnn

SEQ ID NO: 45 - RNA, 100 nt, synthetic construct; identical to SEQ ID NO: 44
  source 1..100: mol_type = other RNA
  modified_base join(1,2): mod_base = OTHER; note = 3-Phosphorothioated 2-OMe-G
  modified_base 3: mod_base = OTHER; note = 3-Phosphorothioated 2-OMe-A
  modified_base join(4,5,8,28,32,34,35,38,46,49,50,55,56,57,58,59,65,69,82,84,87,88,92,94,95,97,98): mod_base = OTHER; note = 2-OMe-A
  modified_base join(6,7,31,47,52,53,61,71,75,81,83): mod_base = um
  modified_base join(9,10,27,29,33,54,60,62,63,68,70,73,74,76,85,89,99,100): mod_base = gm
  modified_base join(11,17,25,90,91,96): mod_base = OTHER; note = 2-Fluoro-U
  modified_base join(12,14,18): mod_base = OTHER; note = 2-Fluoro-G
  modified_base 13: mod_base = OTHER; note = 2-Fluoro-C
  modified_base 15: mod_base = OTHER; note = 3-Phosphorothioated C
  modified_base join(16,22,23,24): mod_base = OTHER; note = 3-Phosphorothioated U
  modified_base 19: mod_base = OTHER; note = 3-Phosphorothioated G
  modified_base join(20,30,42,48,51,64,66,67,72,86): mod_base = cm
  modified_base 77: mod_base = OTHER; note = 3-Phosphorothioated 2-OMe-C
  modified_base join(78,79,80): mod_base = OTHER; note = 3-Phosphorothioated 2-OMe-U
  modified_base join(26,93): mod_base = OTHER; note = 2-Fluoro-A
  modified_base 21: mod_base = OTHER; note = BNA (NC-N-Me)-G

SEQ ID NO: 46 - RNA, 100 nt, synthetic construct; identical to SEQ ID NO: 44
  source 1..100: mol_type = other RNA
  modified_base join(1,2): mod_base = OTHER; note = 3-Phosphorothioated 2-OMe-G
  modified_base 3: mod_base = OTHER; note = 3-Phosphorothioated 2-OMe-A
  modified_base join(4,5,8,28,32,34,35,38,46,49,50,55,56,57,58,59,65,69,82,84,87,88,92,94,95,97,98): mod_base = OTHER; note = 2-OMe-A
  modified_base join(6,7,31,47,52,53,61,71,75,81,83): mod_base = um
  modified_base join(9,10,27,29,33,54,60,62,63,68,70,73,74,76,85,89,99,100): mod_base = gm
  modified_base join(11,17,25,90,91,96): mod_base = OTHER; note = 2-Fluoro-U
  modified_base join(12,14,18): mod_base = OTHER; note = 2-Fluoro-G
  modified_base 13: mod_base = OTHER; note = 2-Fluoro-C
  modified_base 15: mod_base = OTHER; note = 3-Phosphorothioated C
  modified_base join(16,22,23,24): mod_base = OTHER; note = 3-Phosphorothioated U
  modified_base 19: mod_base = OTHER; note = 3-Phosphorothioated G
  modified_base join(20,30,42,48,51,64,66,67,72,86): mod_base = cm
  modified_base 77: mod_base = OTHER; note = 3-Phosphorothioated 2-OMe-C
  modified_base join(78,79,80): mod_base = OTHER; note = 3-Phosphorothioated 2-OMe-U
  modified_base join(26,93): mod_base = OTHER; note = 2-Fluoro-A
  modified_base 21: mod_base = OTHER; note = 2-MOE-G

SEQ ID NO: 47 - RNA, 25 nt, synthetic construct
  source 1..25: mol_type = other RNA
gggaagactatactttcagggatca

SEQ ID NO: 48 - RNA, 21 nt, synthetic construct
  source 1..21: mol_type = other RNA
tttctatagtgtgttactaga

SEQ ID NO: 49 - RNA, 24 nt, synthetic construct
  source 1..24: mol_type = other RNA
gaagtttctctgaacgtgtagagc

SEQ ID NO: 50 - RNA, 21 nt, synthetic construct
  source 1..21: mol_type = other RNA
accgaaaaccacgaggaagag

SEQ ID NO: 51 - RNA, 25 nt, synthetic construct
  source 1..25: mol_type = other RNA
aggtagcgttttctcctgagcgtga

SEQ ID NO: 52 - RNA, 19 nt, synthetic construct
  source 1..19: mol_type = other RNA
agccggctttctggcgttg

SEQ ID NO: 53 - RNA, 25 nt, synthetic construct
  source 1..25: mol_type = other RNA
cttggctgcaactgccgtcagccat

SEQ ID NO: 54 - RNA, 19 nt, synthetic construct
  source 1..19: mol_type = other RNA
tgatgatcgttcttctctc

SEQ ID NO: 55 - RNA, 25 nt, synthetic construct
  source 1..25: mol_type = other RNA
cgtattggggagtgagagggagaga

SEQ ID NO: 56 - RNA, 16 nt, synthetic construct
  source 1..16: mol_type = other RNA
acgcggtctgagtggt

SEQ ID NO: 57 - DNA, 18 bp, synthetic construct
  source 1..18: mol_type = other DNA
tgaaagtatagtcttccc

SEQ ID NO: 58 - DNA, 33 bp, synthetic construct
  source 1..33: mol_type = other DNA
acttctctagtaacacactatagaaatgatccc

SEQ ID NO: 59 - DNA, 12 bp, synthetic construct
  source 1..12: mol_type = other DNA
acgttcagagaa

SEQ ID NO: 60 - DNA, 33 bp, synthetic construct
  source 1..33: mol_type = other DNA
tacctctcttcctcgtggttttcggtgctctac

SEQ ID NO: 61 - DNA, 12 bp, synthetic construct
  source 1..12: mol_type = other DNA
aggagaaaacgc

SEQ ID NO: 62 - DNA, 32 bp, synthetic construct
  source 1..32: mol_type = other DNA
ccaagcaacgccagaaagccggcttcacgctc

SEQ ID NO: 63 - DNA, 13 bp, synthetic construct
  source 1..13: mol_type = other DNA
acggcagttgcag

SEQ ID NO: 64 - DNA, 32 bp, synthetic construct
  source 1..32: mol_type = other DNA
aatacggagagaagaacgatcatcaatggctg

SEQ ID NO: 65 - DNA, 12 bp, synthetic construct
  source 1..12: mol_type = other DNA
ctctcactcccc

SEQ ID NO: 66 - DNA, 23 bp, synthetic construct
  source 1..23: mol_type = other DNA
accactcagaccgcgttctctcc

SEQ ID NO: 67 - DNA, 18 bp, synthetic construct
  source 1..18: mol_type = other DNA
tgaaagtatagtcttccc

SEQ ID NO: 68 - DNA, 33 bp, synthetic construct; identical to SEQ ID NO: 58
  source 1..33: mol_type = other DNA

SEQ ID NO: 69 - DNA, 12 bp, synthetic construct
  source 1..12: mol_type = other DNA
acgttcagagaa

SEQ ID NO: 70 - DNA, 33 bp, synthetic construct; identical to SEQ ID NO: 60
  source 1..33: mol_type = other DNA

SEQ ID NO: 71 - DNA, 12 bp, synthetic construct
  source 1..12: mol_type = other DNA
aggagaaaacgc

SEQ ID NO: 72 - DNA, 32 bp, synthetic construct; identical to SEQ ID NO: 62
  source 1..32: mol_type = other DNA

SEQ ID NO: 73 - DNA, 13 bp, synthetic construct
  source 1..13: mol_type = other DNA
acggcagttgcag

SEQ ID NO: 74 - DNA, 32 bp, synthetic construct; identical to SEQ ID NO: 64
  source 1..32: mol_type = other DNA

SEQ ID NO: 75 - DNA, 12 bp, synthetic construct
  source 1..12: mol_type = other DNA
ctctcactcccc

SEQ ID NO: 76 - DNA, 23 bp, synthetic construct
  source 1..23: mol_type = other DNA
accactcagaccgcgttctctcc

SEQ ID NO: 77 - DNA, 13 bp, synthetic construct
  source 1..13: mol_type = other DNA
tgaaagtatagtc

SEQ ID NO: 78 - DNA, 33 bp, synthetic construct; identical to SEQ ID NO: 58
  source 1..33: mol_type = other DNA

SEQ ID NO: 79 - DNA, 12 bp, synthetic construct
  source 1..12: mol_type = other DNA
acgttcagagaa

SEQ ID NO: 80 - DNA, 33 bp, synthetic construct; identical to SEQ ID NO: 60
  source 1..33: mol_type = other DNA

SEQ ID NO: 81 - DNA, 12 bp, synthetic construct
  source 1..12: mol_type = other DNA
aggagaaaacgc

SEQ ID NO: 82 - DNA, 32 bp, synthetic construct; identical to SEQ ID NO: 62
  source 1..32: mol_type = other DNA

SEQ ID NO: 83 - DNA, 13 bp, synthetic construct
  source 1..13: mol_type = other DNA
acggcagttgcag

SEQ ID NO: 84 - DNA, 32 bp, synthetic construct; identical to SEQ ID NO: 64
  source 1..32: mol_type = other DNA

SEQ ID NO: 85 - DNA, 12 bp, synthetic construct
  source 1..12: mol_type = other DNA
ctctcactcccc

SEQ ID NO: 86 - DNA, 18 bp, synthetic construct
  source 1..18: mol_type = other DNA
tcagaccgcgttctctcc

SEQ ID NO: 87 - DNA, 33 bp, synthetic construct; identical to SEQ ID NO: 58
  source 1..33: mol_type = other DNA

SEQ ID NO: 88 - DNA, 33 bp, synthetic construct; identical to SEQ ID NO: 60
  source 1..33: mol_type = other DNA

SEQ ID NO: 89 - DNA, 32 bp, synthetic construct; identical to SEQ ID NO: 62
  source 1..32: mol_type = other DNA

SEQ ID NO: 90 - DNA, 32 bp, synthetic construct; identical to SEQ ID NO: 64
  source 1..32: mol_type = other DNA

SEQ ID NO: 91 - DNA, 23 bp, synthetic construct
  source 1..23: mol_type = other DNA
accactcagaccgcgttctctcc

SEQ ID NO: 92 - DNA, 18 bp, synthetic construct
  source 1..18: mol_type = other DNA
ctatagaaatgatccctg

SEQ ID NO: 93 - DNA, 18 bp, synthetic construct
  source 1..18: mol_type = other DNA
agaaacttctctagtaac

SEQ ID NO: 94 - DNA, 18 bp, synthetic construct
  source 1..18: mol_type = other DNA
gttttcggtgctctacac

SEQ ID NO: 95 - DNA, 18 bp, synthetic construct
  source 1..18: mol_type = other DNA
acgctacctctcttcctc

SEQ ID NO: 96 - DNA, 18 bp, synthetic construct
  source 1..18: mol_type = other DNA
aagccggcttcacgctca

SEQ ID NO: 97 - DNA, 18 bp, synthetic construct
  source 1..18: mol_type = other DNA
gcagccaagcaacgccag

SEQ ID NO: 98 - DNA, 18 bp, synthetic construct
  source 1..18: mol_type = other DNA
cgatcatcaatggctgac

SEQ ID NO: 99 - DNA, 18 bp, synthetic construct
  source 1..18: mol_type = other DNA
cccaatacggagagaaga

SEQ ID NO: 100 - DNA, 18 bp, synthetic construct
  source 1..18: mol_type = other DNA
agaccgcgttctctccct

SEQ ID NO: 101 - DNA, 16 bp, synthetic construct
  source 1..16: mol_type = other DNA
gaaagtatagtcttcc

SEQ ID NO: 102 - DNA, 31 bp, synthetic construct
  source 1..31: mol_type = other DNA
cttctctagtaacacactatagaaatgatcc

SEQ ID NO: 103 - DNA, 10 bp, synthetic construct
  source 1..10: mol_type = other DNA
cgttcagaga

SEQ ID NO: 104 - DNA, 31 bp, synthetic construct
  source 1..31: mol_type = other DNA
acctctcttcctcgtggttttcggtgctcta

SEQ ID NO: 105 - DNA, 10 bp, synthetic construct
  source 1..10: mol_type = other DNA
ggagaaaacg

SEQ ID NO: 106 - DNA, 30 bp, synthetic construct
  source 1..30: mol_type = other DNA
caagcaacgccagaaagccggcttcacgct

SEQ ID NO: 107 - DNA, 11 bp, synthetic construct
  source 1..11: mol_type = other DNA
cggcagttgca

SEQ ID NO: 108 - DNA, 30 bp, synthetic construct
  source 1..30: mol_type = other DNA
atacggagagaagaacgatcatcaatggct

SEQ ID NO: 109 - DNA, 10 bp, synthetic construct
  source 1..10: mol_type = other DNA
tctcactccc

SEQ ID NO: 110 - DNA, 21 bp, synthetic construct
  source 1..21: mol_type = other DNA
ccactcagaccgcgttctctc

SEQ ID NO: 111 - RNA, 25 nt, synthetic construct
  source 1..25: mol_type = other RNA
ggcaatccggtactgttggtaaagc

SEQ ID NO: 112 - RNA, 15 nt, synthetic construct
  source 1..15: mol_type = other RNA
caccatggtcttcac

SEQ ID NO: 113 - RNA, 25 nt, synthetic construct
  source 1..25: mol_type = other RNA
actcgaagatttcgttggggactgg

SEQ ID NO: 114 - RNA, 15 nt, synthetic construct
  source 1..15: mol_type = other RNA
cgacagacagccggc

SEQ ID NO: 115 - RNA, 27 nt, synthetic construct
  source 1..27: mol_type = other RNA
tacaacctggaccaagtccttgaacag

SEQ ID NO: 116 - RNA, 13 nt, synthetic construct
  source 1..13: mol_type = other RNA
ggaggtgtgtcca

SEQ ID NO: 117 - RNA, 25 nt, synthetic construct
  source 1..25: mol_type = other RNA
gtttgtttcagaatctcggggtgtc

SEQ ID NO: 118 - RNA, 15 nt, synthetic construct
  source 1..15: mol_type = other RNA
cgtaactccgatcca

SEQ ID NO: 119 - RNA, 26 nt, synthetic construct
  source 1..26: mol_type = other RNA
aaggattgtcctgagcggtgaaaatg

SEQ ID NO: 120 - RNA, 14 nt, synthetic construct
  source 1..14: mol_type = other RNA
ggctgaagatcgac

SEQ ID NO: 121 - RNA, 26 nt, synthetic construct
  source 1..26: mol_type = other RNA
atccatgtcatcatcccgtatgaagg

SEQ ID NO: 122 - RNA, 15 nt, synthetic construct
  source 1..15: mol_type = other RNA
tctgagcggcgacca

SEQ ID NO: 123 - RNA, 30 nt, synthetic construct
  source 1..30: mol_type = other RNA
aatgggccagatcgaaaaaatttttaaggt

SEQ ID NO: 124 - RNA, 12 nt, synthetic construct
  source 1..12: mol_type = other RNA
ggtgtaccctgt

SEQ ID NO: 125 - RNA, 19 nt, synthetic construct
  source 1..19: mol_type = other RNA
ggatgatcatcactttaag

SEQ ID NO: 126 - RNA, 18 nt, synthetic construct
  source 1..18: mol_type = other RNA
gtgatcctgcactatggc

SEQ ID NO: 127 - RNA, 25 nt, synthetic construct
  source 1..25: mol_type = other RNA
acactggtaatcgacggggttacgc

SEQ ID NO: 128 - RNA, 15 nt, synthetic construct
  source 1..15: mol_type = other RNA
cgaacatgatcgact

SEQ ID NO: 129 - RNA, 25 nt, synthetic construct
  source 1..25: mol_type = other RNA
atttcggacggccgtatgaaggcat

SEQ ID NO: 130 - RNA, 14 nt, synthetic construct
  source 1..14: mol_type = other RNA
cgccgtgttcgacg

SEQ ID NO: 131 - RNA, 24 nt, synthetic construct
  source 1..24: mol_type = other RNA
gcaaaaagatcactgtaacaggga

SEQ ID NO: 132 - RNA, 16 nt, synthetic construct
  source 1..16: mol_type = other RNA
ccctgtggaacggcaa

SEQ ID NO: 133 - RNA, 26 nt, synthetic construct
  source 1..26: mol_type = other RNA
caaaattatcgacgagcgcctgatca

SEQ ID NO: 134 - RNA, 16 nt, synthetic construct
  source 1..16: mol_type = other RNA
accccgacggctccct

SEQ ID NO: 135 - RNA, 24 nt, synthetic construct
  source 1..24: mol_type = other RNA
gctgttccgagtaaccatcaacgg

SEQ ID NO: 136 - RNA, 13 nt, synthetic construct
  source 1..13: mol_type = other RNA
agtgaccggctgg

SEQ ID NO: 137 - RNA, 27 nt, synthetic construct
  source 1..27: mol_type = other RNA
cggctgtgcgaacgcattctggcgtaa

SEQ ID NO: 138 - RNA, 15 nt, synthetic construct
  source 1..15: mol_type = other RNA
ttctagagtcggggc

SEQ ID NO: 139 - DNA, 20 bp, synthetic construct
  source 1..20: mol_type = other DNA
accaacagtaccggattgcc

SEQ ID NO: 140 - DNA, 25 bp, synthetic construct
  source 1..25: mol_type = other DNA
cgagtgtgaagaccatggtggcttt

SEQ ID NO: 141 - DNA, 15 bp, synthetic construct
  source 1..15: mol_type = other DNA
ccccaacgaaatctt

SEQ ID NO: 142 - DNA, 26 bp, synthetic construct
  source 1..26: mol_type = other DNA
gttgtagccggctgtctgtcgccagt

SEQ ID NO: 143 - DNA, 14 bp, synthetic construct
  source 1..14: mol_type = other DNA
aggacttggtccag

SEQ ID NO: 144 - DNA, 25 bp, synthetic construct
  source 1..25: mol_type = other DNA
caaactggacacacctccctgttca

SEQ ID NO: 145 - DNA, 15 bp, synthetic construct
  source 1..15: mol_type = other DNA
cccgagattctgaaa

SEQ ID NO: 146 - DNA, 25 bp, synthetic construct
  source 1..25: mol_type = other DNA
tcctttggatcggagttacggacac

SEQ ID NO: 147 - DNA, 14 bp, synthetic construct
  source 1..14: mol_type = other DNA
accgctcaggacaa

SEQ ID NO: 148 - DNA, 26 bp, synthetic construct
  source 1..26: mol_type = other DNA
tggatgtcgatcttcagcccattttc

SEQ ID NO: 149 - DNA, 13 bp, synthetic construct
  source 1..13: mol_type = other DNA
cgggatgatgaca

SEQ ID NO: 150 - DNA, 28 bp, synthetic construct
  source 1..28: mol_type = other DNA
ccatttggtcgccgctcagaccttcata

SEQ ID NO: 151 - DNA, 19 bp, synthetic construct
  source 1..19: mol_type = other DNA
aaaattttttcgatctggc

SEQ ID NO: 152 - DNA, 23 bp, synthetic construct
  source 1..23: mol_type = other DNA
catccacagggtacaccacctta

SEQ ID NO: 153 - DNA, 19 bp, synthetic construct
  source 1..19: mol_type = other DNA
atcaccttaaagtgatgat

SEQ ID NO: 154 - DNA, 18 bp, synthetic construct
  source 1..18: mol_type = other DNA
agtgtgccatagtgcagg

SEQ ID NO: 155 - DNA, 15 bp, synthetic construct
  source 1..15: mol_type = other DNA
accccgtcgattacc

SEQ ID NO: 156 - DNA, 26 bp, synthetic construct
  source 1..26: mol_type = other DNA
cgaaatagtcgatcatgttcggcgta

SEQ ID NO: 157 - DNA, 14 bp, synthetic construct
  source 1..14: mol_type = other DNA
ttcatacggccgtc

SEQ ID NO: 158 - DNA, 25 bp, synthetic construct
  source 1..25: mol_type = other DNA
ttttgccgtcgaacacggcgatgcc

SEQ ID NO: 159 - DNA, 13 bp, synthetic construct
  source 1..13: mol_type = other DNA
gttacagtgatct

SEQ ID NO: 160 - DNA, 27 bp, synthetic construct
  source 1..27: mol_type = other DNA
attttgttgccgttccacagggtccct

SEQ ID NO: 161 - DNA, 15 bp, synthetic construct
  source 1..15: mol_type = other DNA
aggcgctcgtcgata

SEQ ID NO: 162 - DNA, 26 bp, synthetic construct
  source 1..26: mol_type = other DNA
acagcagggagccgtcggggttgatc

SEQ ID NO: 163 - DNA, 14 bp, synthetic construct
  source 1..14: mol_type = other DNA
gatggttactcgga

SEQ ID NO: 164 - DNA, 23 bp, synthetic construct
  source 1..23: mol_type = other DNA
agccgccagccggtcactccgtt

SEQ ID NO: 165 - DNA, 17 bp, synthetic construct
  source 1..17: mol_type = other DNA
ccagaatgcgttcgcac

SEQ ID NO: 166 - DNA, 20 bp, synthetic construct
  source 1..20: mol_type = other DNA
gccccgactctagaattacg

SEQ ID NO: 167 - RNA, 25 nt, synthetic construct
  source 1..25: mol_type = other RNA
gggaagactatactttcagggatca

SEQ ID NO: 168 - RNA, 21 nt, synthetic construct
  source 1..21: mol_type = other RNA
tttctatagtgtgttactaga

SEQ ID NO: 169 - RNA, 24 nt, synthetic construct
  source 1..24: mol_type = other RNA
gaagtttctctgaacgtgtagagc

SEQ ID NO: 170 - RNA, 21 nt, synthetic construct
  source 1..21: mol_type = other RNA
accgaaaaccacgaggaagag

SEQ ID NO: 171 - RNA, 25 nt, synthetic construct
  source 1..25: mol_type = other RNA
aggtagcgttttctcctgagcgtga

SEQ ID NO: 172 - RNA, 19 nt, synthetic construct
  source 1..19: mol_type = other RNA
agccggctttctggcgttg

SEQ ID NO: 173 - RNA, 25 nt, synthetic construct
  source 1..25: mol_type = other RNA
cttggctgcaactgccgtcagccat

SEQ ID NO: 174 - RNA, 19 nt, synthetic construct
  source 1..19: mol_type = other RNA
tgatgatcgttcttctctc

SEQ ID NO: 175 - RNA, 25 nt, synthetic construct
  source 1..25: mol_type = other RNA
cgtattggggagtgagagggagaga

SEQ ID NO: 176 - RNA, 16 nt, synthetic construct
  source 1..16: mol_type = other RNA
acgcggtctgagtggt

SEQ ID NO: 177 - RNA, 46 nt, synthetic construct
  source 1..46: mol_type = other RNA
gggaagactatactttcagggatcatttctatagtgtgttactaga

SEQ ID NO: 178 - RNA, 45 nt, synthetic construct
  source 1..45: mol_type = other RNA
tttctatagtgtgttactagagaagtttctctgaacgtgtagagc

SEQ ID NO: 179 - DNA, 18 bp, synthetic construct
  source 1..18: mol_type = other DNA
tgaaagtatagtcttccc

SEQ ID NO: 180 - DNA, 33 bp, synthetic construct; identical to SEQ ID NO: 58
  source 1..33: mol_type = other DNA

SEQ ID NO: 181 - DNA, 12 bp, synthetic construct
  source 1..12: mol_type = other DNA
acgttcagagaa

SEQ ID NO: 182 - DNA, 33 bp, synthetic construct; identical to SEQ ID NO: 60
  source 1..33: mol_type = other DNA

SEQ ID NO: 183 - DNA, 12 bp, synthetic construct
  source 1..12: mol_type = other DNA
aggagaaaacgc

SEQ ID NO: 184 - DNA, 32 bp, synthetic construct; identical to SEQ ID NO: 62
  source 1..32: mol_type = other DNA

SEQ ID NO: 185 - DNA, 13 bp, synthetic construct
  source 1..13: mol_type = other DNA
acggcagttgcag

SEQ ID NO: 186 - DNA, 32 bp, synthetic construct; identical to SEQ ID NO: 64
  source 1..32: mol_type = other DNA

SEQ ID NO: 187 - DNA, 12 bp, synthetic construct
  source 1..12: mol_type = other DNA
ctctcactcccc

SEQ ID NO: 188 - DNA, 23 bp, synthetic construct
  source 1..23: mol_type = other DNA
accactcagaccgcgttctctcc

SEQ ID NO: 189 - DNA, 16 bp, synthetic construct
  source 1..16: mol_type = other DNA
gaaagtatagtcttcc

SEQ ID NO: 190 - DNA, 31 bp, synthetic construct; identical to SEQ ID NO: 102
  source 1..31: mol_type = other DNA

SEQ ID NO: 191 - DNA, 10 bp, synthetic construct
  source 1..10: mol_type = other DNA
cgttcagaga

SEQ ID NO: 192 - DNA, 31 bp, synthetic construct; identical to SEQ ID NO: 104
  source 1..31: mol_type = other DNA

SEQ ID NO: 193 - DNA, 10 bp, synthetic construct
  source 1..10: mol_type = other DNA
ggagaaaacg

SEQ ID NO: 194 - DNA, 30 bp, synthetic construct; identical to SEQ ID NO: 106
  source 1..30: mol_type = other DNA

SEQ ID NO: 195 - DNA, 11 bp, synthetic construct
  source 1..11: mol_type = other DNA
cggcagttgca

SEQ ID NO: 196 - DNA, 30 bp, synthetic construct; identical to SEQ ID NO: 108
  source 1..30: mol_type = other DNA

SEQ ID NO: 197 - DNA, 10 bp, synthetic construct
  source 1..10: mol_type = other DNA
tctcactccc

SEQ ID NO: 198 - DNA, 21 bp, synthetic construct
  source 1..21: mol_type = other DNA
ccactcagaccgcgttctctc

SEQ ID NO: 199 - DNA, 18 bp, synthetic construct
  source 1..18: mol_type = other DNA
ctatagaaatgatccctg

SEQ ID NO: 200 - DNA, 18 bp, synthetic construct
  source 1..18: mol_type = other DNA
agaaacttctctagtaac

SEQ ID NO: 201 - DNA, 18 bp, synthetic construct
  source 1..18: mol_type = other DNA
gttttcggtgctctacac

SEQ ID NO: 202 - DNA, 18 bp, synthetic construct
  source 1..18: mol_type = other DNA
acgctacctctcttcctc

SEQ ID NO: 203 - DNA, 18 bp, synthetic construct
  source 1..18: mol_type = other DNA
aagccggcttcacgctca

SEQ ID NO: 204 - DNA, 18 bp, synthetic construct
  source 1..18: mol_type = other DNA
gcagccaagcaacgccag

SEQ ID NO: 205 - DNA, 18 bp, synthetic construct
  source 1..18: mol_type = other DNA
cgatcatcaatggctgac

SEQ ID NO: 206 - DNA, 18 bp, synthetic construct
  source 1..18: mol_type = other DNA
cccaatacggagagaaga

SEQ ID NO: 207 - DNA, 18 bp, synthetic construct
  source 1..18: mol_type = other DNA
agaccgcgttctctccct

SEQ ID NO: 208 - DNA, 16 bp, synthetic construct
  source 1..16: mol_type = other DNA
aaagtatagtcttccc

SEQ ID NO: 209 - DNA, 19 bp, synthetic construct
  source 1..19: mol_type = other DNA
actatagaaatgatccctg

SEQ ID NO: 210 - DNA, 23 bp, synthetic construct
  source 1..23: mol_type = other DNA
cagagaaacttctctagtaacac

SEQ ID NO: 211 - DNA, 23 bp, synthetic construct
  source 1..23: mol_type = other DNA
tggttttcggtgctctacacgtt

SEQ ID NO: 212 - DNA, 23 bp, synthetic construct
  source 1..23: mol_type = other DNA
gaaaacgctacctctcttcctcg

SEQ ID NO: 213 - DNA, 22 bp, synthetic construct
  source 1..22: mol_type = other DNA
aaagccggcttcacgctcagga

SEQ ID NO: 214 - DNA, 21 bp, synthetic construct
  source 1..21: mol_type = other DNA
gttgcagccaagcaacgccag

SEQ ID NO: 215 - DNA, 22 bp, synthetic construct
  source 1..22: mol_type = other DNA
cgatcatcaatggctgacggca

SEQ ID NO: 216 - DNA, 23 bp, synthetic construct
  source 1..23: mol_type = other DNA
actccccaatacggagagaagaa

SEQ ID NO: 217 - DNA, 21 bp, synthetic construct
  source 1..21: mol_type = other DNA
agaccgcgttctctccctctc

SEQ ID NO: 218 - skipped

SEQ ID NO: 219 - DNA, 78 bp, synthetic construct
  source 1..78: mol_type = other DNA
tacctctcttcctcgtggttttcggtgctctacacgttcagagaaacttctctagtaacacactatagaaatgatccc

SEQ ID NO: 220 - RNA, 25 nt, synthetic construct
  source 1..25: mol_type = other RNA
gggaggtctatataagcagagctcg

SEQ ID NO: 221 - RNA, 16 nt, synthetic construct
  source 1..16: mol_type = other RNA
tttagtgaaccgtcag

SEQ ID NO: 222 - RNA, 24 nt, synthetic construct
  source 1..24: mol_type = other RNA
atcactagaagctttattgcggta

SEQ ID NO: 223 - RNA, 16 nt, synthetic construct
  source 1..16: mol_type = other RNA
gtttatcacagttaaa

SEQ ID NO: 224 - RNA, 20 nt, synthetic construct
  source 1..20: mol_type = other RNA
ttgctaacgcagtcagtggg

SEQ ID NO: 225 - RNA, 17 nt, synthetic construct
  source 1..17: mol_type = other RNA
cctcggcggccaagctt

SEQ ID NO: 226 - RNA, 32 nt, synthetic construct
  source 1..32: mol_type = other RNA
gcttcgagcagacatgataagatacattgatg

SEQ ID NO: 227 - RNA, 27 nt, synthetic construct
  source 1..27: mol_type = other RNA
agtttggacaaaccacaactagaatgc

SEQ ID NO: 228 - RNA, 24 nt, synthetic construct
  source 1..24: mol_type = other RNA
agtgaaaaaaatgctttatttgtg

SEQ ID NO: 229 - RNA, 21 nt, synthetic construct
  source 1..21: mol_type = other RNA
aaatttgtgatgctattgctt

SEQ ID NO: 230 - RNA, 31 nt, synthetic construct
  source 1..31: mol_type = other RNA
ggcaatccggtactgttggtaaagccaccat

SEQ ID NO: 231 - RNA, 537 nt, synthetic construct
  source 1..537: mol_type = other RNA
ggtcttcacactcgaagatttcgttggggactggcgacagacagccggctacaacctggaccaagtccttgaacagggaggtgtgtccagtttgtttcagaatctcggggtgtccgtaactccgatccaaaggattgtcctgagcggtgaaaatgggctgaagatcgacatccatgtcatcatcccgtatgaaggtctgagcggcgaccaaatgggccagatcgaaaaaatttttaaggtggtgtaccctgtggatgatcatcactttaaggtgatcctgcactatggcacactggtaatcgacggggttacgccgaacatgatcgactatttcggacggccgtatgaaggcatcgccgtgttcgacggcaaaaagatcactgtaacagggaccctgtggaacggcaacaaaattatcgacgagcgcctgatcaaccccgacggctccctgctgttccgagtaaccatcaacggagtgaccggctggcggctgtgcgaacgcattctggcgtaattctagagtcggggcggccggcc

SEQ ID NO: 232 - DNA, 20 bp, synthetic construct
  source 1..20: mol_type = other DNA
tctgcttatatagacctccc

SEQ ID NO: 233 - DNA, 26 bp, synthetic construct
  source 1..26: mol_type = other DNA
gtgatctgacggttcactaaacgagc

SEQ ID NO: 234 - DNA, 14 bp, synthetic construct
  source 1..14: mol_type = other DNA
caataaagcttcta

SEQ ID NO: 235 - DNA, 26 bp, synthetic construct
  source 1..26: mol_type = other DNA
agcaatttaactgtgataaactaccg

SEQ ID NO: 236 - DNA, 20 bp, synthetic construct
  source 1..20: mol_type = other DNA
cgaggcccactgactgcgtt

SEQ ID NO: 237 - DNA, 17 bp, synthetic construct
  source 1..17: mol_type = other DNA
ttgccaagcttggccgc

SEQ ID NO: 238 - DNA, 38 bp, synthetic construct
  source 1..38: mol_type = other DNA
tcactgcattctagttgtggtttgtccaaactcatcaa

SEQ ID NO: 239 - DNA, 13 bp, synthetic construct
  source 1..13: mol_type = other DNA
taaagcatttttt

SEQ ID NO: 240 - DNA, 27 bp, synthetic construct
  source 1..27: mol_type = other DNA
aagcaatagcatcacaaatttcacaaa

SEQ ID NO: 241 - DNA, 15 bp, synthetic construct
  source 1..15: mol_type = other DNA
accaacagtaccgga

SEQ ID NO: 242 - DNA, 54 bp, synthetic construct
  source 1..54: mol_type = other DNA
tgtatcttatcatgtctgctcgaagcggccggccgccccgactctagaattacg

SEQ ID NO: 243 - RNA, 34 nt, synthetic construct
  source 1..34: mol_type = other RNA
ggtcttcacactcgaagatttcgttggggactgg